European Patent Specification EP 4 240 842 B1, published December 18, 2024. Title: TARGETED SEQUENCING METHOD AND KIT THEREOF FOR DETECTING GENE ALTERATION. Applicant: ACT GENOMICS CO., LTD. The sequence listing filed with the application follows.

SEQUENCE LISTING (36 sequences)

SEQ ID NO: 1 - DNA, 19 bp, Artificial Sequence
  Synthesized Primer
gttttcccagtcacgacgt

SEQ ID NO: 2 - DNA, 21 bp, Artificial Sequence
  Synthesized Primer
gcaaatggcattctgacatcc

SEQ ID NO: 3 - DNA, 22 bp, Artificial Sequence
  Synthesized Primer
gcggataacaatttcacacagg

SEQ ID NO: 4 - DNA, 17 bp, Artificial Sequence
  Synthesized Primer
cgtccatgccgagagtg

SEQ ID NO: 5 - DNA, 23 bp, Artificial Sequence
  Synthesized Primer
ctttatgtttttggcgtcttcca

SEQ ID NO: 6 - DNA, 21 bp, Artificial Sequence
  Synthesized Primer
gactggttccaattgacaagc

SEQ ID NO: 7 - DNA, 19 bp, Artificial Sequence
  Synthesized Primer
gcgtgaatgtaagcgtgac

SEQ ID NO: 8 - DNA, 18 bp, Artificial Sequence
  Synthesized Primer
tgtaaaacgacggccagt

SEQ ID NO: 9 - DNA, 20 bp, Artificial Sequence
  Synthesized Primer
aagggtcttgcgaaggatag

SEQ ID NO: 10 - DNA, 23 bp, Artificial Sequence
  Synthesized Primer
gggttatgctagttattgctcag

SEQ ID NO: 11 - DNA, 26 bp, Artificial Sequence
  Synthesized Primer
aagagaaagcaaattaaagatcagtt

SEQ ID NO: 12 - DNA, 19 bp, Artificial Sequence
  Synthesized Primer
ctgtcagaggatactgcac

SEQ ID NO: 13 - DNA, 40 bp, Artificial Sequence
  MET-MET fusion
aaagagaaagcaaattaaagatcagtttcctaattcatct

SEQ ID NO: 14 - DNA, 17 bp, Artificial Sequence
  Synthesized Primer
atgtcagcgtttggctt

SEQ ID NO: 15 - DNA, 20 bp, Artificial Sequence
  Synthesized Primer
tttcgtccttcttctccacc

SEQ ID NO: 16 - DNA, 20 bp, Artificial Sequence
  Synthesized Primer
ccacatcatggtctctgtct

SEQ ID NO: 17 - DNA, 17 bp, Artificial Sequence
  Synthesized Primer
ggctgagtcctcctcac

SEQ ID NO: 18 - DNA, 17 bp, Artificial Sequence
  Synthesized Primer
cagccggaggtcatact

SEQ ID NO: 19 - DNA, 17 bp, Artificial Sequence
  Synthesized Primer
ggctgagtcctcctcac

SEQ ID NO: 20 - DNA, 21 bp, Artificial Sequence
  Synthesized Primer
ccagctacatcaatccttgag

SEQ ID NO: 21 - DNA, 20 bp, Artificial Sequence
  Synthesized Primer
ctggcagagtcatcatcatt

SEQ ID NO: 22 - protein, 19 aa, Artificial Sequence
  Synthesized Primer
ACAGCAGCCACCATATACA

SEQ ID NO: 23 - DNA, 18 bp, Artificial Sequence
  Synthesized Primer
aggtgtttcgtccttctt

SEQ ID NO: 24 - DNA, 20 bp, Artificial Sequence
  Synthesized Primer
tggcttaacagatgatcagg

SEQ ID NO: 25 - DNA, 17 bp, Artificial Sequence
  Synthesized Primer
gagaaggggatgcacca

SEQ ID NO: 26 - DNA, 17 bp, Artificial Sequence
  Synthesized Primer
gacccgtgctgagtttg

SEQ ID NO: 27 - DNA, 17 bp, Artificial Sequence
  Synthesized Primer
cagcccatcctctggag

SEQ ID NO: 28 - DNA, 21 bp, Artificial Sequence
  Synthesized Primer
gaggtcatactgcatcagaac

SEQ ID NO: 29 - DNA, 21 bp, Artificial Sequence
  Synthesized Primer
cattggagatgtgatggagtg

SEQ ID NO: 30 - DNA, 17 bp, Artificial Sequence
  Synthesized Primer
tccccgcctgaagagca

SEQ ID NO: 31 - DNA, 17 bp, Artificial Sequence
  Synthesized Primer
tctcgcttcagcacgat

SEQ ID NO: 32 - DNA, 21 bp, Artificial Sequence
  Synthesized Primer
accatatacaggagctcagac

SEQ ID NO: 33 - DNA, 17 bp, Artificial Sequence
  Synthesized Primer
ctcgatgcagtgctcca

SEQ ID NO: 34 - DNA, 19 bp, Artificial Sequence
  Synthesized Primer
gggctctggaggaaaagaa

SEQ ID NO: 35 - DNA, 19 bp, Artificial Sequence
  Synthesized Primer
tccatctcatagctgtcgg

SEQ ID NO: 36 - DNA, 40 bp, Artificial Sequence
  EGFR-EGFR fusion
gctctggaggaaaagaaagttgtggtgacagatcacggct